European Patent Specification EP 4 009 957 B1, published October 11, 2023. Title: SOLID COMPOSITION COMPRISING A PYY COMPOUND AND A SALT OF N-(8-(2-HYDROXYBENZOYL)AMINO)CAPRYLIC ACID. Applicant: NOVO NORDISK A/S. The sequence listing filed with the application follows.

SEQUENCE LISTING (34 sequences)

SEQ ID NO: 1 - protein, 36 aa, HOMO SAPIENS
  MISC_FEATURE: hPYY(1-36)
  MISC_FEATURE (36)..(36): AMIDATION
YPIKPEAPGEDASPEELNRYYASLRHYLNLVTRQRY

SEQ ID NO: 2 - protein, 34 aa, HOMO SAPIENS
  MISC_FEATURE: hPYY(3-36)
  MISC_FEATURE (34)..(34): AMIDATION
IKPEAPGEDASPEELNRYYASLRHYLNLVTRQRY

SEQ ID NO: 3 - protein, 34 aa, ARTIFICIAL
  Artificial protein based on human PYY
  MISC_FEATURE (34)..(34): AMIDATION
IRPEKPGEDASPEELQRYYASLRHYYNWLTRQRY

SEQ ID NO: 4 - protein, 33 aa, ARTIFICIAL
  Artificial protein based on human PYY
  MISC_FEATURE (33)..(33): AMIDATION
RPEKPGEDASPEELQRYYASLRHYYNWLTRQRY

SEQ ID NO: 5 - protein, 33 aa, ARTIFICIAL
  Artificial protein based on human PYY
  MISC_FEATURE (33)..(33): AMIDATION
RPEKPPEDASPEELQRYYASLRHYYNWLTRQRY

SEQ ID NO: 6 - protein, 33 aa, ARTIFICIAL
  Artificial protein based on human PYY
  MISC_FEATURE (33)..(33): AMIDATION
RPEKPSEDASPEELQRYYASLRHYYNWLTRQRY

SEQ ID NO: 7 - protein, 33 aa, ARTIFICIAL
  Artificial protein based on human PYY
  MISC_FEATURE (33)..(33): AMIDATION
RPEKPTEDASPEELQRYYASLRHYYNWLTRQRY

SEQ ID NO: 8 - protein, 33 aa, ARTIFICIAL
  Artificial protein based on human PYY
  MISC_FEATURE (33)..(33): AMIDATION
RPEKPGEDATPEELQRYYASLRHYYNWLTRQRY

SEQ ID NO: 9 - protein, 33 aa, ARTIFICIAL
  Artificial protein based on human PYY
  MISC_FEATURE (33)..(33): AMIDATION
RPEKPGEDASPEELQRYYASARHYYNWLTRQRY

SEQ ID NO: 10 - protein, 33 aa, ARTIFICIAL
  Artificial protein based on human PYY
  MISC_FEATURE (33)..(33): AMIDATION
RPEKPGEDASPEELQRYYASIRHYYNWLTRQRY

SEQ ID NO: 11 - protein, 34 aa, ARTIFICIAL
  Artificial protein based on human PYY
  MISC_FEATURE (34)..(34): AMIDATION
ZRPEKPGEDASPEELQRYYASIRHYYNWLTRQRY

SEQ ID NO: 12 - protein, 34 aa, ARTIFICIAL
  Artificial protein based on human PYY
  MISC_FEATURE (34)..(34): AMIDATION
IRPEKPGEDASPEELQRYYISLRHYLNWLTRQRY

SEQ ID NO: 13 - protein, 33 aa, ARTIFICIAL
  Artificial protein based on human PYY
  MISC_FEATURE (33)..(33): AMIDATION
RPEKPGEDASPEELQRYYISLRHYLNWLTRQRY

SEQ ID NO: 14 - protein, 33 aa, ARTIFICIAL
  Artificial protein based on human PYY
  MISC_FEATURE (33)..(33): AMIDATION
RPEKPPEDASPEELQRYYISLRHYLNWLTRQRY

SEQ ID NO: 15 - protein, 33 aa, ARTIFICIAL
  Artificial protein based on human PYY
  MISC_FEATURE (33)..(33): AMIDATION
RPEKPGEDASPEELQRYYISLRHYYNWLTRQRY

SEQ ID NO: 16 - protein, 33 aa, ARTIFICIAL
  Artificial protein based on human PYY
  MISC_FEATURE (33)..(33): AMIDATION
RPEKPGEDASPEELQRYYISARHYYNWLTRQRY

SEQ ID NO: 17 - protein, 33 aa, ARTIFICIAL
  Artificial protein based on human PYY
  MISC_FEATURE (33)..(33): AMIDATION
RPEKPGEDASPEELQRYYQSLRHYYNWLTRQRY

SEQ ID NO: 18 - protein, 33 aa, ARTIFICIAL
  Artificial protein based on human PYY
  MISC_FEATURE (33)..(33): AMIDATION
RPEKPGEDASPEELQRYYVSLRHYYNWLTRQRY

SEQ ID NO: 19 - protein, 33 aa, ARTIFICIAL
  Artificial protein based on human PYY
  MISC_FEATURE (33)..(33): AMIDATION
RPEKPTEDASPEELQRYYQSLRHYYNWLTRQRY

SEQ ID NO: 20 - protein, 33 aa, ARTIFICIAL
  Artificial protein based on human PYY
  MISC_FEATURE (33)..(33): AMIDATION
RPEKPTEDASPEELQRYYVSLRHYYNWLTRQRY

SEQ ID NO: 21 - protein, 33 aa, ARTIFICIAL
  Artificial protein based on human PYY
  MISC_FEATURE (33)..(33): AMIDATION
RPEKPGEDATPEELQRYYQSLRHYYNWLTRQRY

SEQ ID NO: 22 - protein, 33 aa, ARTIFICIAL
  Artificial protein based on human PYY
  MISC_FEATURE (33)..(33): AMIDATION
RPEKPGEDATPEELQRYYVSLRHYYNWLTRQRY

SEQ ID NO: 23 - protein, 33 aa, Artificial Sequence
  Artificial protein based on human PYY
  MISC_FEATURE (33)..(33): Amidation
RPEAPGKDASPEELQRYYESLRHYYNWLTRQRY

SEQ ID NO: 24 - protein, 33 aa, Artificial Sequence
  Artificial protein based on human PYY
  MISC_FEATURE (33)..(33): Amidation
RPEAPGKDASPEELQRYYAELRHYYNWLTRQRY

SEQ ID NO: 25 - protein, 33 aa, Artificial Sequence
  Artificial protein based on human PYY
  MISC_FEATURE (33)..(33)
  MOD_RES (33)..(33): AMIDATION
RPEAPPKDASPEELQRYYESLRHYYNWLTRQRY

SEQ ID NO: 26 - protein, 33 aa, Artificial Sequence
  Artificial protein based on human PYY
  MOD_RES (33)..(33): AMIDATION
RPEAPPKDASPEELQRYYASLRHYYNWLTRQRY

SEQ ID NO: 27 - protein, 33 aa, Artificial Sequence
  Artificial protein based on human PYY
  MOD_RES (33)..(33): AMIDATION
RPEAPGKDASPEELQRYYASLRHYYNWLTRQRY

SEQ ID NO: 28 - protein, 33 aa, Artificial Sequence
  Artificial protein based on human PYY
  MOD_RES (33)..(33): AMIDATION
RPEAPGEDASPEELQRYYASLRHYYNWLTRQRY

SEQ ID NO: 29 - protein, 33 aa, Homo sapiens
  MISC_FEATURE: hPYY(4-36)
  MISC_FEATURE (33)..(33): AMIDATION
KPEAPGEDASPEELNRYYASLRHYLNLVTRQRY

SEQ ID NO: 30 - protein, 30 aa, Homo sapiens
  MISC_FEATURE: GLP-1(7-36)
HAEGTFTSDVSSYLEGQAAKEFIAWLVKGR

SEQ ID NO: 31 - protein, 31 aa, Homo sapiens
  MISC_FEATURE: GLP-1(7-37)
HAEGTFTSDVSSYLEGQAAKEFIAWLVKGRG

SEQ ID NO: 32 - protein, 31 aa, Artificial Sequence
  Synthetic petide
  MISC_FEATURE: Semaglutide
  MISC_FEATURE (2)..(2): X is alpha-aminoisobutyric acid (Aib)
HXEGTFTSDVSSYLEGQAAKEFIAWLVRGRG

SEQ ID NO: 33 - protein, 33 aa, Artificial Sequence
  Synthetic peptide
  MISC_FEATURE: GLP-1 agonist A
  MISC_FEATURE (2)..(2): X is alpha-aminoisobutyric acid (Aib)
HXEGTFTSDVSSYLEEQAARKFIEWLVRGKGEG

SEQ ID NO: 34 - protein, 29 aa, Homo sapiens
HSQGTFTSDYSKYLDSRRAQDFVQWLMNT